European Patent Application EP 4 534 099 A1, published April 9, 2025. Title: ＩＬ－１２ｐ７０を恒常的に産生する増殖性ミエロイド細胞の製造方法. Applicant: 北京天一方生物科技发展有限公司. The sequence listing filed with the application follows.

SEQUENCE LISTING (32 sequences)

SEQ ID NO: 1 - DNA, 711 bp, Mus musculus
  source 1..711: mol_type = other DNA
atggtcagcgttccaacagcctcaccctcggcatccagcagctcctctcagtgccggtccagcatgtgtcaatcacgctacctcctctttttggccacccttgccctcctaaaccacctcagtttggccagggtcattccagtctctggacctgccaggtgtcttagccagtcccgaaacctgctgaagaccacagatgacatggtgaagacggccagagaaaaactgaaacattattcctgcactgctgaagacatcgatcatgaagacatcacacgggaccaaaccagcacattgaagacctgtttaccactggaactacacaagaacgagagttgcctggctactagagagacttcttccacaacaagagggagctgcctgcccccacagaagacgtctttgatgatgaccctgtgccttggtagcatctatgaggacttgaagatgtaccagacagagttccaggccatcaacgcagcacttcagaatcacaaccatcagcagatcattctagacaagggcatgctggtggccatcgatgagctgatgcagtctctgaatcataatggcgagactctgcgccagaaacctcctgtgggagaagcagacccttacagagtgaaaatgaagctctgcatcctgcttcacgccttcagcacccgcgtcgtgaccatcaacagggtgatgggctatctgagctccgcctga

SEQ ID NO: 2 - DNA, 1008 bp, Mus musculus
  source 1..1008: mol_type = other DNA
atgtgtcctcagaagctaaccatctcctggtttgccatcgttttgctggtgtctccactcatggccatgtgggagctggagaaagacgtttatgttgtagaggtggactggactcccgatgcccctggagaaacagtgaacctcacctgtgacacgcctgaagaagatgacatcacctggacctcagaccagagacatggagtcataggctctggaaagaccctgaccatcactgtcaaagagtttctagatgctggccagtacacctgccacaaaggaggcgagactctgagccactcacatctgctgctccacaagaaggaaaatggaatttggtccactgaaattttaaaaaatttcaaaaacaagactttcctgaagtgtgaagcaccaaattactccggacggttcacgtgctcatggctggtgcaaagaaacatggacttgaagttcaacatcaagagcagtagcagttcccctgactctcgggcagtgacatgtggaatggcgtctctgtctgcagagaaggtcacactggaccaaagggactatgagaagtattcagtgtcctgccaggaggatgtcacctgcccaactgccgaggagaccctgcccattgaactggcgttggaagcacggcagcagaataaatatgagaactacagcaccagcttcttcatcagggacatcatcaaaccagacccgcccaagaacttgcagatgaagcctttgaagaactcacaggtggaggtcagctgggagtaccctgactcctggagcactccccattcctacttctccctcaagttctttgttcgaatccagcgcaagaaagaaaagatgaaggagacagaggaggggtgtaaccagaaaggtgcgttcctcgtagagaagacatctaccgaagtccaatgcaaaggcgggaatgtctgcgtgcaagctcaggatcgctattacaattcctcatgcagcaagtgggcatgtgttccctgcagggtccgatcctag

SEQ ID NO: 3 - DNA, 54 bp, Thosea asigna virus
  source 1..54: mol_type = other DNA
gagggcagaggcagcctgctgacctgcggcgacgtggaggaaaaccctggccct

SEQ ID NO: 4 - DNA, 1320 bp, Homo sapiens
  source 1..1320: mol_type = other DNA
atgcccctcaacgttagcttcaccaacaggaactatgacctcgactacgactcggtgcagccgtatttctactgcgacgaggaggagaacttctaccagcagcagcagcagagcgagctgcagcccccggcgcccagcgaggatatctggaagaaattcgagctgctgcccaccccgcccctgtcccctagccgccgctccgggctctgctcgccctcctacgttgcggtcacacccttctcccttcggggagacaacgacggcggtggcgggagcttctccacggccgaccagctggagatggtgaccgagctgctgggaggagacatggtgaaccagagtttcatctgcgacccggacgacgagaccttcatcaaaaacatcatcatccaggactgtatgtggagcggcttctcggccgccgccaagctcgtctcagagaagctggcctcctaccaggctgcgcgcaaagacagcggcagcccgaaccccgcccgcggccacagcgtctgctccacctccagcttgtacctgcaggatctgagcgccgccgcctcagagtgcatcgacccctcggtggtcttcccctaccctctcaacgacagcagctcgcccaagtcctgcgcctcgcaagactccagcgccttctctccgtcctcggattctctgctctcctcgacggagtcctccccgcagggcagccccgagcccctggtgctccatgaggagacaccgcccaccaccagcagcgactctgaggaggaacaagaagatgaggaagaaatcgatgttgtttctgtggaaaagaggcaggctcctggcaaaaggtcagagtctggatcaccttctgctggaggccacagcaaacctcctcacagcccactggtcctcaagaggtgccacgtctccacacatcagcacaactacgcagcgcctccctccactcggaaggactatcctgctgccaagagggtcaagttggacagtgtcagagtcctgagacagatcagcaacaaccgaaaatgcaccagccccaggtcctcggacaccgaggagaatgtcaagaggcgaacacacaacgtcttggagcgccagaggaggaacgagctaaaacggagcttttttgccctgcgtgaccagatcccggagttggaaaacaatgaaaaggcccccaaggtagttatccttaaaaaagccacagcatacatcctgtccgtccaagcagaggagcaaaagctcatttctgaagaggacttgttgcggaaacgacgagaacagttgaaacacaaacttgaacagctacggaactcttgtgcgtaa

SEQ ID NO: 5 - DNA, 981 bp, Homo sapiens
  source 1..981: mol_type = other DNA
atgcatcgaacaacgagaatcaagatcactgagctaaatccccacctgatgtgtgtgctttgtggagggtacttcattgatgccacaaccataatagaatgtctacattccttctgtaaaacgtgtattgttcgttacctggagaccagcaagtattgtcctatttgtgatgtccaagttcacaagaccagaccactactgaatataaggtcagataaaactctccaagatattgtatacaaattagttccagggcttttcaaaaatgaaatgaagagaagaagggatttttatgcagctcatccttctgctgatgctgccaatggctctaatgaagatagaggagaggttgcagatgaagataagagaattataactgatgatgagataataagcttatccattgaattctttgaccagaacagattggatcggaaagtaaacaaagacaaagagaaatctaaggaggaggtgaatgataaaagatacttacgatgcccagcagcaatgactgtgatgcacttaagaaagtttctcagaagtaaaatggacatacctaatactttccagattgatgtcatgtatgaggaggaacctttaaaggattattatacactaatggatattgcctacatttatacctggagaaggaatggtccacttccattgaaatacagagttcgacctacttgtaaaagaatgaagatcagtcaccagagagatggactgacaaatgctggagaactggaaagtgactctgggagtgacaaggccaacagcccagcaggaggtattccctccacctcttcttgtttgcctagccccagtactccagtgcagtctcctcatccacagtttcctcacatttccagtactatgaatggaaccagcaacagccccagcggtaaccaccaatcttcttttgccaatagacctcgaaaatcatcagtaaatgggtcatcagcaacttcttctggttga

SEQ ID NO: 6 - DNA, 1494 bp, Homo sapiens
  source 1..1494: mol_type = other DNA
atggtgaggagcaggcaaatgtgcaataccaacatgtctgtacctactgatggtgctgtaaccacctcacagattccagcttcggaacaagagaccctggttagaccaaagccattgcttttgaagttattaaagtctgttggtgcacaaaaagacacttatactatgaaagaggttcttttttatcttggccagtatattatgactaaacgattatatgatgagaagcaacaacatattgtatattgttcaaatgatcttctaggagatttgtttggcgtgccaagcttctctgtgaaagagcacaggaaaatatataccatgatctacaggaacttggtagtagtcaatcagcaggaatcatcggactcaggtacatctgtgagtgagaacaggtgtcaccttgaaggtgggagtgatcaaaaggaccttgtacaagagcttcaggaagagaaaccttcatcttcacatttggtttctagaccatctacctcatctagaaggagagcaattagtgagacagaagaaaattcagatgaattatctggtgaacgacaaagaaaacgccacaaatctgatagtatttccctttcctttgatgaaagcctggctctgtgtgtaataagggagatatgttgtgaaagaagcagtagcagtgaatctacagggacgccatcgaatccggatcttgatgctggtgtaagtgaacattcaggtgattggttggatcaggattcagtttcagatcagtttagtgtagaatttgaagttgaatctctcgactcagaagattatagccttagtgaagaaggacaagaactctcagatgaagatgatgaggtatatcaagttactgtgtatcaggcaggggagagtgatacagattcatttgaagaagatcctgaaatttccttagctgactattggaaatgcacttcatgcaatgaaatgaatcccccccttccatcacattgcaacagatgttgggcccttcgtgagaattggcttcctgaagataaagggaaagataaaggggaaatctctgagaaagccaaactggaaaactcaacacaagctgaagagggctttgatgttcctgattgtaaaaaaactatagtgaatgattccagagagtcatgtgttgaggaaaatgatgataaaattacacaagcttcacaatcacaagaaagtgaagactattctcagccatcaacttctagtagcattatttatagcagccaagaagatgtgaaagagtttgaaagggaagaaacccaagacaaagaagagagtgtggaatctagtttgccccttaatgccattgaaccttgtgtgatttgtcaaggtcgacctaaaaatggttgcattgtccatggcaaaacaggacatcttatggcctgctttacatgtgcaaagaagctaaagaaaaggaataagccctgcccagtatgtagacaaccaattcaaatgattgtgctaacttatttcccctag

SEQ ID NO: 7 - DNA, 8872 bp, synthetic construct
  misc_feature 1..8872: note = pSL plasmid vector
  source 1..8872: mol_type = other DNA
tcgcgcgtttcggtgatgacggtgaaaacctctgacacatgcagctcccggagacggtcacagcttgtctgtaagcggatgccgggagcagacaagcccgtcagggcgcgtcagcgggtgttggcgggtgtcggggctggcttaactatgcggcatcagagcagattgtactgagagtgcaccatatgcggtgtgaaataccgcacagatgcgtaaggagaaaataccgcatcaggcgccattcgccattcaggctgcgcaactgttgggaagggcgatcggtgcgggcctcttcgctattacgccagctggcgaaagggggatgtgctgcaaggcgattaagttgggtaacgccagggttttcccagtcacgacgttgtaaaacgacggccagtgaattcgacggatcgggagatctcccgatcccctatggtcgactctcagtacaatctgctctgatgccgcatagttaagccagtatctgctccctgcttgtgtgttggaggtcgctgagtagtgcgcgagcaaaatttaagctacaacaaggcaaggcttgaccgacaattgcatgaagaatctgcttagggttaggcgttttgcgctgcttcgcgatgtacgggccagatatacgcgttgacattgattattgactagttattaatagtaatcaattacggggtcattagttcatagcccatatatggagttccgcgttacataacttacggtaaatggcccgcctggctgaccgcccaacgacccccgcccattgacgtcaataatgacgtatgttcccatagtaacgccaatagggactttccattgacgtcaatgggtggagtatttacggtaaactgcccacttggcagtacatcaagtgtatcatatgccaagtacgccccctattgacgtcaatgacggtaaatggcccgcctggcattatgcccagtacatgaccttatgggactttcctacttggcagtacatctacgtattagtcatcgctattaccatggtgatgcggttttggcagtacatcaatgggcgtggatagcggtttgactcacggggatttccaagtctccaccccattgacgtcaatgggagtttgttttggcaccaaaatcaacgggactttccaaaatgtcgtaacaactccgccccattgacgcaaatgggcggtaggcgtgtacggtgggaggtctatataagcagcgcgttttgcctgtactgggtctctctggttagaccagatctgagcctgggagctctctggctaactagggaacccactgcttaagcctcaataaagcttgccttgagtgcttcaagtagtgtgtgcccgtctgttgtgtgactctggtaactagagatccctcagacccttttagtcagtgtggaaaatctctagcagtggcgcccgaacagggacttgaaagcgaaagggaaaccagaggagctctctcgacgcaggactcggcttgctgaagcgcgcacggcaagaggcgaggggcggcgactggtgagtacgccaaaaattttgactagcggaggctagaaggagagagatgggtgcgagagcgtcagtattaagcgggggagaattagatcgcgatgggaaaaaattcggttaaggccagggggaaagaaaaaatataaattaaaacatatagtatgggcaagcagggagctagaacgattcgcagttaatcctggcctgttagaaacatcagaaggctgtagacaaatactgggacagctacaaccatcccttcagacaggatcagaagaacttagatcattatataatacagtagcaaccctctattgtgtgcatcaaaggatagagataaaagacaccaaggaagctttagacaagatagaggaagagcaaaacaaaagtaagaccaccgcacagcaagcggccggccgctgatcttcagacctggaggaggagatatgagggacaattggagaagtgaattatataaatataaagtagtaaaaattgaaccattaggagtagcacccaccaaggcaaagagaagagtggtgcagagagaaaaaagagcagtgggaataggagctttgttccttgggttcttgggagcagcaggaagcactatgggcgcagcgtcaatgacgctgacggtacaggccagacaattattgtctggtatagtgcagcagcagaacaatttgctgagggctattgaggcgcaacagcatctgttgcaactcacagtctggggcatcaagcagctccaggcaagaatcctggctgtggaaagatacctaaaggatcaacagctcctggggatttggggttgctctggaaaactcatttgcaccactgctgtgccttggaatgctagttggagtaataaatctctggaacagatttggaatcacacgacctggatggagtgggacagagaaattaacaattacacaagcttaatacactccttaattgaagaatcgcaaaaccagcaagaaaagaatgaacaagaattattggaattagataaatgggcaagtttgtggaattggtttaacataacaaattggctgtggtatataaaattattcataatgatagtaggaggcttggtaggtttaagaatagtttttgctgtactttctatagtgaatagagttaggcagggatattcaccattatcgtttcagacccacctcccaaccccgaggggacccgacaggcccgaaggaatagaagaagaaggtggagagagagacagagacagatccattcgattagtgaacggatctacaaatggcagtattcatccacaattttaaaagaaaaggggggattggggggtacagtgcaggggaaagaatagtagacataatagcaacagacatacaaactaaagaattacaaaaacaaattacaaaaattcaaaattttcgggtttattacagggacagcagaaattcactttgaattaattcaagcttcgtgaggctccggtgcccgtcagtgggcagagcgcacatcgcccacagtccccgagaagttggggggaggggtcggcaattgaaccggtgcctagagaaggtggcgcggggtaaactgggaaagtgatgtcgtgtactggctccgcctttttcccgagggtgggggagaaccgtatataagtgcagtagtcgccgtgaacgttctttttcgcaacgggtttgccgccagaacacaggtaagtgccgtgtgtggttcccgcgggcctggcctctttacgggttatggcccttgcgtgccttgaattacttccacctggctccagtacgtgattcttgatcccgagctggagccaggggcgggccttgcgctttaggagccccttcgcctcgtgcttgagttgaggcctggcctgggcgctggggccgccgcgtgcgaatctggtggcaccttcgcgcctgtctcgctgctttcgataagtctctagccatttaaaatttttgatgacctgctgcgacgctttttttctggcaagatagtcttgtaaatgcgggccaggatctgcacactggtatttcggtttttggggccgcgggcggcgacggggcccgtgcgtcccagcgcacatgttcggcgaggcggggcctgcgagcgcggccaccgagaatcggacgggggtagtctcaagctggccggcctgctctggtgcctggcctcgcgccgccgtgtatcgccccgccctgggcggcaaggctggcccggtcggcaccagttgcgtgagcggaaagatggccgcttcccggccctgctccagggggctcaaaatggaggacgcggcgctcgggagagcgggcgggtgagtcacccacacaaaggaaaggggcctttccgtcctcagccgtcgcttcatgtgactccacggagtaccgggcgccgtccaggcacctcgattagttctggagcttttggagtacgtcgtctttaggttggggggaggggttttatgcgatggagtttccccacactgagtgggtggagactgaagttaggccagcttggcacttgatgtaattctccttggaatttgccctttttgagtttggatcttggttcattctcaagcctcagacagtggttcaaagtttttttcttccatttcaggtgtcgtgaacacgctaccggtctcgagaattctgcagcggccgcggatcctctagagttaacatcgagggatcaagcttatcgataatcaacctctggattacaaaatttgtgaaagattgactggtattcttaactatgttgctccttttacgctatgtggatacgctgctttaatgcctttgtatcatgctattgcttcccgtatggctttcattttctcctccttgtataaatcctggttgctgtctctttatgaggagttgtggcccgttgtcaggcaacgtggcgtggtgtgcactgtgtttgctgacgcaacccccactggttggggcattgccaccacctgtcagctcctttccgggactttcgctttccccctccctattgccacggcggaactcatcgccgcctgccttgcccgctgctggacaggggctcggctgttgggcactgacaattccgtggtgttgtcggggaagctgacgtcctttccatggctgctcgcctgtgttgccacctggattctgcgcgggacgtccttctgctacgtcccttcggccctcaatccagcggaccttccttcccgcggcctgctgccggctctgcggcctcttccgcgtcttcgccttcgccctcagacgagtcggatctccctttgggccgcctccccgcatcgataccgtcgagacctggaaaaacatggagcaatcacaagtagcaacacagcagctaccaatgctgcttgtgcctggctagaagcacaagaggaggaggaggtgggttttccagtcacacctcaggtacctttaagaccaatgacttacaaggcagctgtagatcttagccactttttaaaagaaaaggggggactggaagggctaattcactcccaacgaagacaagatatccttgatctgtggatctaccacacacaaggctacttccctgattggcagaactacacaccagggccagggatcagatatccactgacctttggatggtgctacaagctagtaccagttgagcaagagaaggtagaagaagccaatgaaggagagaacacccgcttgttacaccctgtgagcctgcatgggatggatgacccggagagagaagtattagagtggaggtttgacagccgcctagcatttcatcacatggcccgagagctgcatccggactgtactgggtctctctggttagaccagatctgagcctgggagctctctggctaactagggaacccactgcttaagcctcaataaagcttgccttgagtgcttcaagtagtgtgtgcccgtctgttgtgtgactctggtaactagagatccctcagacccttttagtcagtgtggaaaatctctagcagggcccgtttaaacccgctgatcagcctcgactgtgccttctagttgccagccatctgttgtttgcccctcccccgtgccttccttgaccctggaaggtgccactcccactgtcctttcctaataaaatgaggaaattgcatcgcattgtctgagtaggtgtcattctattctggggggtggggtggggcaggacagcaagggggaggattgggaagacaatagcaggcatgctggggatgcggtgggctctatggcttctgaggcggaaagaaccagctggggctctagggggtatccccacgcgccctgtagcggcgcattaagcgcggcgggtgtggtggttacgcgcagcgtgaccgctacacttgccagcgccctagcgcccgctcctttcgctttcttcccttcctttctcgccacgttcgccggctttccccgtcaagctctaaatcggggcatccctttagggttccgatttagtgctttacggcacctcgaccccaaaaaacttgattagggtgatggttcacgtagtgggccatcgccctgatagacggtttttcgccctttgacgttggagtccacgttctttaatagtggactcttgttccaaactggaacaacactcaaccctatctcggtctattcttttgatttataagggattttggggatttcggcctattggttaaaaaatgagctgatttaacaaaaatttaacgcgaattaattctgtggaatgtgtgtcagttagggtgtggaaagtccccaggctccccaggcaggcagaagtatgcaaagcatgcatctcaattagtcagcaaccaggtgtggaaagtccccaggctccccagcaggcagaagtatgcaaagcatgcatctcaattagtcagcaaccatagtcccgcccctaactccgcccatcccgcccctaactccgcccagttccgcccattctccgccccatggctgactaattttttttatttatgcagaggccgaggccgcctctgcctctgagctattccagaagtagtgaggaggcttttttggaggcctaggcttttgcaaaaagctcccgggagcttgtatatccattttcgcctgcatgcaagcttggcgtaatcatggtcatagctgtttcctgtgtgaaattgttatccgctcacaattccacacaacatacgagccggaagcataaagtgtaaagcctggggtgcctaatgagtgagctaactcacattaattgcgttgcgctcactgcccgctttccagtcgggaaacctgtcgtgccagctgcattaatgaatcggccaacgcgcggggagaggcggtttgcgtattgggcgctcttccgcttcctcgctcactgactcgctgcgctcggtcgttcggctgcggcgagcggtatcagctcactcaaaggcggtaatacggttatccacagaatcaggggataacgcaggaaagaacatgtgagcaaaaggccagcaaaaggccaggaaccgtaaaaaggccgcgttgctggcgtttttccataggctccgcccccctgacgagcatcacaaaaatcgacgctcaagtcagaggtggcgaaacccgacaggactataaagataccaggcgtttccccctggaagctccctcgtgcgctctcctgttccgaccctgccgcttaccggatacctgtccgcctttctcccttcgggaagcgtggcgctttctcatagctcacgctgtaggtatctcagttcggtgtaggtcgttcgctccaagctgggctgtgtgcacgaaccccccgttcagcccgaccgctgcgccttatccggtaactatcgtcttgagtccaacccggtaagacacgacttatcgccactggcagcagccactggtaacaggattagcagagcgaggtatgtaggcggtgctacagagttcttgaagtggtggcctaactacggctacactagaagaacagtatttggtatctgcgctctgctgaagccagttaccttcggaaaaagagttggtagctcttgatccggcaaacaaaccaccgctggtagcggtggtttttttgtttgcaagcagcagattacgcgcagaaaaaaaggatctcaagaagatcctttgatcttttctacggggtctgacgctcagtggaacgaaaactcacgttaagggattttggtcatgagattatcaaaaaggatcttcacctagatccttttaaattaaaaatgaagttttaaatcaatctaaagtatatatgagtaaacttggtctgacagttaccaatgcttaatcagtgaggcacctatctcagcgatctgtctatttcgttcatccatagttgcctgactccccgtcgtgtagataactacgatacgggagggcttaccatctggccccagtgctgcaatgataccgcgagacccacgctcaccggctccagatttatcagcaataaaccagccagccggaagggccgagcgcagaagtggtcctgcaactttatccgcctccatccagtctattaattgttgccgggaagctagagtaagtagttcgccagttaatagtttgcgcaacgttgttgccattgctacaggcatcgtggtgtcacgctcgtcgtttggtatggcttcattcagctccggttcccaacgatcaaggcgagttacatgatcccccatgttgtgcaaaaaagcggttagctccttcggtcctccgatcgttgtcagaagtaagttggccgcagtgttatcactcatggttatggcagcactgcataattctcttactgtcatgccatccgtaagatgcttttctgtgactggtgagtactcaaccaagtcattctgagaatagtgtatgcggcgaccgagttgctcttgcccggcgtcaatacgggataataccgcgccacatagcagaactttaaaagtgctcatcattggaaaacgttcttcggggcgaaaactctcaaggatcttaccgctgttgagatccagttcgatgtaacccactcgtgcacccaactgatcttcagcatcttttactttcaccagcgtttctgggtgagcaaaaacaggaaggcaaaatgccgcaaaaaagggaataagggcgacacggaaatgttgaatactcatactcttcctttttcaatattattgaagcatttatcagggttattgtctcatgagcggatacatatttgaatgtatttagaaaaataaacaaataggggttccgcgcacatttccccgaaaagtgccacctgacgtctaagaaaccattattatcatgacattaacctataaaaataggcgtatcacgaggccctttcgtc

SEQ ID NO: 8 - DNA, 762 bp, Homo sapiens
  source 1..762: mol_type = other DNA
atgtggccccctgggtcagcctcccagccaccgccctcacctgccgcggccacaggtctgcatccagcggctcgccctgtgtccctgcagtgccggctcagcatgtgtccagcgcgcagcctcctccttgtggctaccctggtcctcctggaccacctcagtttggccagaaacctccccgtggccactccagacccaggaatgttcccatgccttcaccactcccaaaacctgctgagggccgtcagcaacatgctccagaaggccagacaaactctagaattttacccttgcacttctgaagagattgatcatgaagatatcacaaaagataaaaccagcacagtggaggcctgtttaccattggaattaaccaagaatgagagttgcctaaattccagagagacctctttcataactaatgggagttgcctggcctccagaaagacctcttttatgatggccctgtgccttagtagtatttatgaagacttgaagatgtaccaggtggagttcaagaccatgaatgcaaagcttctgatggaccctaagaggcagatctttctagatcaaaacatgctggcagttattgatgagctgatgcaggccctgaatttcaacagtgagactgtgccacaaaaatcctcccttgaagaaccggatttttataaaactaaaatcaagctctgcatacttcttcatgctttcagaattcgggcagtgactattgatagagtgatgagctatctgaatgcttcctga

SEQ ID NO: 9 - DNA, 987 bp, Homo sapiens
  source 1..987: mol_type = other DNA
atgtgtcaccagcagttggtcatctcttggttttccctggtttttctggcatctcccctcgtggccatatgggaactgaagaaagatgtttatgtcgtagaattggattggtatccggatgcccctggagaaatggtggtcctcacctgtgacacccctgaagaagatggtatcacctggaccttggaccagagcagtgaggtcttaggctctggcaaaaccctgaccatccaagtcaaagagtttggagatgctggccagtacacctgtcacaaaggaggcgaggttctaagccattcgctcctgctgcttcacaaaaaggaagatggaatttggtccactgatattttaaaggaccagaaagaacccaaaaataagacctttctaagatgcgaggccaagaattattctggacgtttcacctgctggtggctgacgacaatcagtactgatttgacattcagtgtcaaaagcagcagaggctcttctgacccccaaggggtgacgtgcggagctgctacactctctgcagagagagtcagaggggacaacaaggagtatgagtactcagtggagtgccaggaggacagtgcctgcccagctgctgaggagagtctgcccattgaggtcatggtggatgccgttcacaagctcaagtatgaaaactacaccagcagcttcttcatcagggacatcatcaaacctgacccacccaagaacttgcagctgaagccattaaagaattctcggcaggtggaggtcagctgggagtaccctgacacctggagtactccacattcctacttctccctgacattctgcgttcaggtccagggcaagagcaagagagaaaagaaagatagagtcttcacggacaagacctcagccacggtcatctgccgcaaaaatgccagcattagcgtgcgggcccaggaccgctactatagctcatcttggagcgaatgggcatctgtgccctgcagttag

SEQ ID NO: 10 - DNA, 57 bp, Porcine teschovirus-1
  source 1..57: mol_type = other DNA
gctactaacttcagcctgctgaagcaggctggagacgtggaggagaaccctggacct

SEQ ID NO: 11 - DNA, 574 bp, Poliovirus
  source 1..574: mol_type = other DNA
cccctctccctcccccccccctaacgttactggccgaagccgcttggaataaggccggtgtgcgtttgtctatatgttattttccaccatattgccgtcttttggcaatgtgagggcccggaaacctggccctgtcttcttgacgagcattcctaggggtctttcccctctcgccaaaggaatgcaaggtctgttgaatgtcgtgaaggaagcagttcctctggaagcttcttgaagacaaacaacgtctgtagcgaccctttgcaggcagcggaaccccccacctggcgacaggtgcctctgcggccaaaagccacgtgtataagatacacctgcaaaggcggcacaaccccagtgccacgttgtgagttggatagttgtggaaagagtcaaatggctctcctcaagcgtattcaacaaggggctgaaggatgcccagaaggtaccccattgtatgggatctgatctggggcctcggtgcacatgctttacatgtgtttagtcgaggttaaaaaaacgtctaggccccccgaaccacggggacgtggttttcctttgaaaaacacgatgataa

SEQ ID NO: 12 - DNA, 1002 bp, Homo sapiens
  source 1..1002: mol_type = other DNA
atgccacctcctcgcctcctcttcttcctcctcttcctcacccctatggaagtcaggcccgaggaacctctagtggtgaaggtggaagagggagataacgctgtgctgcagtgcctcaaggggacctcagatggccccactcagcagctgacctggtctcgggagtccccgcttaaacccttcttaaaactcagcctggggctgccaggcctgggaatccacatgaggcccctggccatctggcttttcatcttcaacgtctctcaacagatggggggcttctacctgtgccagccgggacccccctctgagaaggcctggcagcctggctggacagtcaatgtggagggcagcggggagctgttccggtggaatgtttcggacctaggtggcctgggctgtggcctgaagaacaggtcctcagagggacccagctccccttccgggaagctcatgagccccaagctgtatgtgtgggccaaagaccgccctgagatatgggagggagagcctccgtgtctcccaccgagggacagcctgaaccagagcctcagccaggacctcactatggcccctggctccacactctggctgtcctgtggggtaccccctgactctgtgtccaggggacccctctcctggacccatgtgcaccccaaggggcctaagtcattgctgagcctagagctgaaggacgatcgcccggccagagatatgtgggtaatggagacgggtctgttgttgccccgggccacagctcaagacgctggaaagtattattgtcaccgtggcaacctgaccatgtcattccacctggagatcactgctcggccagcactatggcactggctgctgaggactggtggctggaaggtctcagctgtgactttggcttatctgatcttctgcctgtgttcccttgtgggcattcttcatcttcaaagagccctggtcctgaggaggaaaagaaagcgaatgactgaccccaccaggagattctga

SEQ ID NO: 13 - DNA, 20 bp, synthetic construct
  misc_feature 1..20: note = target sequence of gRNA for H- 2Kb and H- 2Db
  source 1..20: mol_type = other DNA
gaatccgagatatgagccgc

SEQ ID NO: 14 - DNA, 20 bp, synthetic construct
  misc_feature 1..20: note = target sequence of gRNA for I-Ab
  source 1..20: mol_type = other DNA
ggctgctgtggtggtgctga

SEQ ID NO: 15 - DNA, 45 bp, synthetic construct
  misc_feature 1..45: note = (G4S)3 linker
  source 1..45: mol_type = other DNA
ggtggcggtggtagcggcggtggcggcagcggtggcggcggcagt

SEQ ID NO: 16 - DNA, 213 bp, Mus musculus
  source 1..213: mol_type = other DNA
cccccagaagaccctcctgatagcaagaacacacttgtgctctttggggcaggattcggcgcagtaataacagtcgtcgtcatcgttgtcatcatcaaatgcttctgtaagcacagaagctgtttcagaagaaatgaggcaagcagagaaacaaacaacagccttaccttcgggcctgaagaagcattagctgaacagaccgtcttcctttag

SEQ ID NO: 17 - DNA, 20 bp, synthetic construct
  misc_feature 1..20: note = target sequence of gRNA for mouse SIRPalpha
  source 1..20: mol_type = other DNA
gggtcccaccggcaacaagg

SEQ ID NO: 18 - DNA, 81 bp, Mus musculus
  source 1..81: mol_type = other DNA
atggcctcaccgttgacccgctttctgtcgctgaacctgctgctgctgggtgagtcgattatcctggggagtggagaagct

SEQ ID NO: 19 - DNA, 348 bp, synthetic construct
  misc_feature 1..348: note = GC33 VH
  source 1..348: mol_type = other DNA
tcccaggtccagttgcagcagtccggtgctgagcttgtgaggcctggcgcttctgtgaaactgtcatgcaaagcatcaggctacacttttaccgattatgagatgcattgggtcaagcagaccccagttcacgggctcaaatggatcggcgccctggaccccaaaactggggacaccgcctactcccaaaagttcaagggaaaggccactctgactgcagacaagagctcctctacagcctatatggaactgcggtctttgaccagtgaagatagcgcagtgtattactgtaccagattctacagttatacatactggggacaaggtacactcgtgacagtaagcgct

SEQ ID NO: 20 - DNA, 75 bp, synthetic construct
  misc_feature 1..75: note = 205c linker
  source 1..75: mol_type = other DNA
agcagcgccgacgacgccaagaaggacgccgccaagaaggacgacgccaagaaggacgacgccaagaaggacggc

SEQ ID NO: 21 - DNA, 339 bp, synthetic construct
  misc_feature 1..339: note = GC33 VL
  source 1..339: mol_type = other DNA
gacgtggtgatgacacagacccccctttctctccccgtgtccctgggtgatcaggctagcatctcctgcagatcctcccagagtctggtgcatagtaacggcaacacatatctgcactggtatctgcaaaaacccggtcagtctccaaaactgctcatctacaaggtttctaatcggttcagcggcgtcccagacaggtttagcgggtctgggagcggcacagactttactttgaagattagtcgcgtcgaggccgaagatttgggcgtttatttctgttcacagaatacccacgtacctcctaccttcggatcaggaactaagcttgagataaagcgg

SEQ ID NO: 22 - DNA, 246 bp, Mus musculus
  source 1..246: mol_type = other DNA
gtcgtgccagtccttcagaaagtgaactctactactaccaagccagtgctgcgaactccctcacctgtgcaccctaccgggacatctcagccccagagaccagaagattgtcggccccgtggctcagtgaaggggaccggattggacttcgcctgtgatatttacatctgggcacccttggccggaatctgcgtggcccctctgctgtccttgatcatcactctcatctgctaccacaggagccga

SEQ ID NO: 23 - DNA, 342 bp, Mus musculus
  source 1..342: mol_type = other DNA
agagcaaaattcagcaggagtgcagagactgctgccaacctgcaggaccccaaccagctctacaatgagctcaatctagggcgaagagaggaatatgacgtcttggagaagaagcgggctcgggacccagagatgggaggcaaacagcagaggaggaggaacccccaggaaggcgtatacaatgcactgcagaaagacaagatggcagaagcctacagtgagatcggcacaaaaggcgagaggcggagaggcaaggggcacgatggcctttaccagggtctcagcactgccaccaaggacacctatgatgccctgcatatgcagaccctggcccctcgctaa

SEQ ID NO: 24 - DNA, 993 bp, Mus musculus
  source 1..993: mol_type = other DNA
atgccatctcctctccctgtctccttcctcctctttcttaccttagtaggaggcaggccccagaagtccttactggtggaggtagaagagggaggcaatgttgtgctgccatgcctcccggactcctcacctgtctcttctgagaagctggcttggtatcgaggtaaccagtcaacacccttcctggagctgagccccgggtcccctggcctgggattgcacgtggggtccctgggcatcttgctagtgattgtcaatgtctcagaccatatggggggcttctacctgtgccagaagaggccccctttcaaggacatctggcagcctgcctggacagtgaacgtggaggatagtggggagatgttccggtggaatgcttcagacgtcagggacctggactgtgacctaaggaacaggtcctctgggagccacaggtccacttctggttcccagctgtatgtgtgggctaaagaccatcctaaggtctggggaacaaagcctgtatgtgcccctcgggggagcagtttgaatcagagtctaatcaaccaagatctcactgtggcacccggctccacactttggctgtcctgtggggtaccccctgtcccagtggccaaaggctccatctcctggacccatgtgcatcctaggagacctaatgtttcactactgagcctaagccttgggggagagcacccggtcagagagatgtgggtttgggggtctcttctgcttctgccccaagccacagctttagatgaaggcacctattattgtctccgaggaaacctgaccatcgagaggcacgtgaaggtcattgcaaggtcagcagtgtggctctggctgttgagaactggtggatggatagtcccagtggtgactttagtatatgtcatcttctgtatggtttctctggtggcttttctctattgtcaaagagcctttatcctgagaaggaaaaggaagcgaatgactgaccccgccaggagattc

SEQ ID NO: 25 - DNA, 20 bp, synthetic construct
  misc_feature 1..20: note = target sequence of gRNA for human HLA-ABC
  source 1..20: mol_type = other DNA
agcaggaggggccggagtat

SEQ ID NO: 26 - DNA, 20 bp, synthetic construct
  misc_feature 1..20: note = target sequence of gRNA for human CIITA
  source 1..20: mol_type = other DNA
ctgccattgcttgaaccgtc

SEQ ID NO: 27 - DNA, 1098 bp, Homo sapiens
  source 1..1098: mol_type = other DNA
atggccgtcatggcgccccgaaccctcgtcctgctactctcgggggctctggccctgacccagacctgggcgggctctcactccatgaggtatttcttcacatccgtgtcccggcccggccgcggggagccccgcttcatcgcagtgggctacgtggacgacacgcagttcgtgcggttcgacagcgacgccgcgagccagaggatggagccgcgggcgccgtggatagagcaggagggtccggagtattgggacggggagacacggaaagtgaaggcccactcacagactcaccgagtggacctggggaccctgcgcggctactacaaccagagcgaggccggttctcacaccgtccagaggatgtatggctgcgacgtggggtcggactggcgcttcctccgcgggtaccaccagtacgcctacgacggcaaggattacatcgccctgaaagaggacctgcgctcttggaccgcggcggacatggcagctcagaccaccaagcacaagtgggaggcggcccatgtggcggagcagttgagagcctacctggagggcacgtgcgtggagtggctccgcagatacctggagaacgggaaggagacgctgcagcgcacggacgcccccaaaacgcatatgactcaccacgctgtctctgaccatgaagccaccctgaggtgctgggccctgagcttctaccctgcggagatcacactgacctggcagcgggatggggaggaccagacccaggacacggagctcgtggagaccaggcctgcaggggatggaaccttccagaagtgggcggctgtggtggtgccttctggacaggagcagagatacacctgccatgtgcagcatgagggtttgcccaagcccctcaccctgagatgggagccgtcttcccagcccaccatccccatcgtgggcatcattgctggcctggttctctttggagctgtgatcactggagctgtggtcgctgctgtgatgtggaggaggaagagctcagatagaaaaggagggagctactctcaggctgcaagcagtgacagtgcccagggctctgatgtgtctctcacagcttgtaaagtgtga

SEQ ID NO: 28 - DNA, 1098 bp, Homo sapiens
  source 1..1098: mol_type = other DNA
atggccgtcatggcgccccgaaccctcgtcctgctactctcgggggccctggccctgacccagacctgggcaggctcccactccatgaggtatttctccacatccgtgtcccggcccggccgcggggagccccgcttcatcgccgtgggctacgtggacgacacgcagttcgtgcggttcgacagcgacgccgcgagccagaggatggagccgcgggcgccgtggatagagcaggaggggccggagtattgggacgaggagacagggaaagtgaaggcccactcacagactgaccgagagaacctgcggatcgcgctccgctactacaaccagagcgaggccggttctcacaccctccagatgatgtttggctgcgacgtggggtcggacgggcgcttcctccgcgggtaccaccagtacgcctacgacggcaaggattacatcgccctgaaagaggacctgcgctcttggaccgcggcggacatggcggctcagatcaccaagcgcaagtgggaggcggcccatgtggcggagcagcagagagcctacctggagggcacgtgcgtggacgggctccgcagatacctggagaacgggaaggagacgctgcagcgcacggacccccccaagacacatatgacccaccaccccatctctgaccatgaggccactctgagatgctgggccctgggcttctaccctgcggagatcacactgacctggcagcgggatggggaggaccagacccaggacacggagcttgtggagaccaggcctgcaggggatggaaccttccagaagtgggcagctgtggtggtaccttctggagaggagcagagatacacctgccatgtgcagcatgagggtctgcccaagcccctcaccctgagatgggagccatcttcccagcccaccgtccccatcgtgggcatcattgctggcctggttctccttggagctgtgatcactggagctgtggtcgctgctgtgatgtggaggaggaacagctcagatagaaaaggagggagctactctcaggctgcaagcagtgacagtgcccagggctctgatgtgtctctcacagcttgtaaagtgtga

SEQ ID NO: 29 - DNA, 147 bp, Homo sapiens
  source 1..147: mol_type = other DNA
gataacctgctcccatcctgggccattaccttaatctcagtaaatggaatttttgtgatatgctgcctgacctactgctttgccccaagatgcagagagagaaggaggaatgagagattgagaagggaaagtgtacgccctgtataa

SEQ ID NO: 30 - DNA, 63 bp, Homo sapiens
  source 1..63: mol_type = other DNA
atggccttaccagtgaccgccttgctcctgccgctggccttgctgctccacgccgccaggccg

SEQ ID NO: 31 - DNA, 249 bp, Homo sapiens
  source 1..249: mol_type = other DNA
ttcgtgcctgtctttctgcccgccaagcctaccacaactccagctcctcgcccccctacaccagcaccaactatcgcctcccagcctctgtctctgcgaccagaggcatgccggcccgcagctggaggagcagtgcacacacggggcctggacttcgcttgcgacatctacatttgggctcccctggctggaacttgtggcgtgctgctgctgagtctggtcattaccctgtactgtaaccacagaaat

SEQ ID NO: 32 - DNA, 339 bp, Homo sapiens
  source 1..339: mol_type = other DNA
agagtcaagtttagcaggtccgctgatgcacccgcctaccagcagggacagaatcagctgtataacgagctgaatctgggcaggcgcgaggaatatgacgtgctggataaacgacgggggagagaccccgaaatggggggaaagcctagaaggaaaaacccacaggagggactgtacaatgaactgcagaaggacaaaatggctgaggcatatagcgaaattgggatgaagggagaacgccgacggggcaaaggacacgatggactgtaccaggggctgtccactgccaccaaggacacctatgatgctctgcatatgcaggcactgcctccacggtaa